European Patent Specification EP 3 824 100 B1, published April 29, 2026. Title: POLYNUCLEOTIDE SYNTHESIS METHOD, KIT AND SYSTEM. Applicant: OXFORD NANOPORE TECHNOLOGIES LIMITED. Application To be assigned. The sequence listing filed with the application follows.

SEQUENCE LISTING (83 sequences)

SEQ ID NO: 1 - DNA, 18 bp, Artificial Sequence
  source: /note="Description of Artificial Sequence: Synthetic primer"
gcgacaggtgactgcagc

SEQ ID NO: 2 - DNA, 36 bp, Artificial Sequence
  source: /note="Description of Artificial Sequence: Synthetic oligonucleotide"
  modified_base (18)..(18): 2'-deoxyinosine
cacatcacgtcgtagtcngctgcagtcacctgtcgc

SEQ ID NO: 3 - DNA, 36 bp, Artificial Sequence; identical to SEQ ID NO: 2
  source: /note="Description of Artificial Sequence: Synthetic oligonucleotide"
  modified_base (18)..(18): 2'-deoxyinosine

SEQ ID NO: 4 - DNA, 19 bp, Artificial Sequence
  source: /note="Description of Artificial Sequence: Synthetic primer"
gcgacaggtgactgcagct

SEQ ID NO: 5 - DNA, 36 bp, Artificial Sequence
  source: /note="Description of Artificial Sequence: Synthetic oligonucleotide"
gcgacaggtgactgcagctgactacgacgtgatgtg

SEQ ID NO: 6 - DNA, 36 bp, Artificial Sequence
  source: /note="Description of Artificial Sequence: Synthetic oligonucleotide"
  modified_base (17)..(17): 2'-deoxyinosine
cacatcacgtcgtagtnagctgcagtcacctgtcgc

SEQ ID NO: 7 - DNA, 18 bp, Artificial Sequence
  source: /note="Description of Artificial Sequence: Synthetic oligonucleotide"
gctgcagtcacctgtcgc

SEQ ID NO: 8 - DNA, 19 bp, Artificial Sequence
  source: /note="Description of Artificial Sequence: Synthetic primer"
gcgacaggtgactgcagct

SEQ ID NO: 9 - DNA, 18 bp, Artificial Sequence
  source: /note="Description of Artificial Sequence: Synthetic oligonucleotide"
  modified_base (17)..(17): 2'-deoxyinosine
cacatcacgtcgtagtna

SEQ ID NO: 10 - DNA, 18 bp, Artificial Sequence
  source: /note="Description of Artificial Sequence: Synthetic primer"
gcgacaggtgactgcagc

SEQ ID NO: 11 - DNA, 36 bp, Artificial Sequence; identical to SEQ ID NO: 2
  source: /note="Description of Artificial Sequence: Synthetic oligonucleotide"
  modified_base (18)..(18): 2'-deoxyinosine

SEQ ID NO: 12 - DNA, 18 bp, Artificial Sequence
  source: /note="Description of Artificial Sequence: Synthetic oligonucleotide"
cgactacgacgtgatgtg

SEQ ID NO: 13 - DNA, 36 bp, Artificial Sequence; identical to SEQ ID NO: 2
  source: /note="Description of Artificial Sequence: Synthetic oligonucleotide"
  modified_base (18)..(18): Deoxyinosine

SEQ ID NO: 14 - DNA, 19 bp, Artificial Sequence
  source: /note="Description of Artificial Sequence: Synthetic primer"
gcgacaggtgactgcagct

SEQ ID NO: 15 - DNA, 36 bp, Artificial Sequence; identical to SEQ ID NO: 5
  source: /note="Description of Artificial Sequence: Synthetic oligonucleotide"

SEQ ID NO: 16 - DNA, 18 bp, Artificial Sequence
  source: /note="Description of Artificial Sequence: Synthetic oligonucleotide"
tgactacgacgtgatgtg

SEQ ID NO: 17 - DNA, 36 bp, Artificial Sequence; identical to SEQ ID NO: 6
  source: /note="Description of Artificial Sequence: Synthetic oligonucleotide"
  modified_base (17)..(17): 2'-deoxyinosine

SEQ ID NO: 18 - DNA, 18 bp, Artificial Sequence
  source: /note="Description of Artificial Sequence: Synthetic oligonucleotide"
gctgcagtcacctgtcgc

SEQ ID NO: 19 - DNA, 19 bp, Artificial Sequence
  source: /note="Description of Artificial Sequence: Synthetic primer"
gcgacaggtgactgcagct

SEQ ID NO: 20 - DNA, 18 bp, Artificial Sequence
  source: /note="Description of Artificial Sequence: Synthetic oligonucleotide"
  modified_base (17)..(17): 2'-deoxyinosine
cacatcacgtcgtagtna

SEQ ID NO: 21 - DNA, 17 bp, Artificial Sequence
  source: /note="Description of Artificial Sequence: Synthetic oligonucleotide"
cactacgacgtgatgtg

SEQ ID NO: 22 - DNA, 18 bp, Artificial Sequence
  source: /note="Description of Artificial Sequence: Synthetic primer"
gcgacaggtgactgcagc

SEQ ID NO: 23 - DNA, 37 bp, Artificial Sequence
  source: /note="Description of Artificial Sequence: Synthetic oligonucleotide"
  modified_base (18)..(18): 2'-deoxyinosine
cacatcacgtcgtagtcnagctgcagtcacctgtcgc

SEQ ID NO: 24 - DNA, 37 bp, Artificial Sequence
  source: /note="Description of Artificial Sequence: Synthetic oligonucleotide"
  modified_base (18)..(18): 2'-deoxyinosine
cacatcacgtcgtagtcnggctgcagtcacctgtcgc

SEQ ID NO: 25 - DNA, 37 bp, Artificial Sequence; identical to SEQ ID NO: 23
  source: /note="Description of Artificial Sequence: Synthetic oligonucleotide"
  modified_base (18)..(18): 2'-deoxyinosine

SEQ ID NO: 26 - DNA, 37 bp, Artificial Sequence; identical to SEQ ID NO: 23
  source: /note="Description of Artificial Sequence: Synthetic oligonucleotide"
  modified_base (18)..(18): 2'-deoxyinosine

SEQ ID NO: 27 - DNA, 19 bp, Artificial Sequence
  source: /note="Description of Artificial Sequence: Synthetic oligonucleotide"
tcgactacgacgtgatgtg

SEQ ID NO: 28 - DNA, 19 bp, Artificial Sequence
  source: /note="Description of Artificial Sequence: Synthetic oligonucleotide"
ccgactacgacgtgatgtg

SEQ ID NO: 29 - DNA, 19 bp, Artificial Sequence
  source: /note="Description of Artificial Sequence: Synthetic oligonucleotide"
acgactacgacgtgatgtg

SEQ ID NO: 30 - DNA, 19 bp, Artificial Sequence
  source: /note="Description of Artificial Sequence: Synthetic oligonucleotide"
gcgactacgacgtgatgtg

SEQ ID NO: 31 - DNA, 37 bp, Artificial Sequence; identical to SEQ ID NO: 23
  source: /note="Description of Artificial Sequence: Synthetic oligonucleotide"
  modified_base (18)..(18): Deoxyinosine

SEQ ID NO: 32 - DNA, 19 bp, Artificial Sequence
  source: /note="Description of Artificial Sequence: Synthetic primer"
gcgacaggtgactgcagct

SEQ ID NO: 33 - DNA, 36 bp, Artificial Sequence; identical to SEQ ID NO: 5
  source: /note="Description of Artificial Sequence: Synthetic oligonucleotide"

SEQ ID NO: 34 - DNA, 19 bp, Artificial Sequence
  source: /note="Description of Artificial Sequence: Synthetic oligonucleotide"
tcgactacgacgtgatgtg

SEQ ID NO: 35 - DNA, 18 bp, Artificial Sequence
  source: /note="Description of Artificial Sequence: Synthetic oligonucleotide"
gctgcagtcacctgtcgc

SEQ ID NO: 36 - DNA, 19 bp, Artificial Sequence
  source: /note="Description of Artificial Sequence: Synthetic primer"
gcgacaggtgactgcagct

SEQ ID NO: 37 - DNA, 19 bp, Artificial Sequence
  source: /note="Description of Artificial Sequence: Synthetic oligonucleotide"
  modified_base (17)..(17): 2'-deoxyinosine
cacatcacgtcgtagtnga

SEQ ID NO: 38 - DNA, 18 bp, Artificial Sequence
  source: /note="Description of Artificial Sequence: Synthetic oligonucleotide"
ccactacgacgtgatgtg

SEQ ID NO: 39 - DNA, 18 bp, Artificial Sequence
  source: /note="Description of Artificial Sequence: Synthetic primer"
gcgacaggtgactgcagc

SEQ ID NO: 40 - DNA, 36 bp, Artificial Sequence
  source: /note="Description of Artificial Sequence: Synthetic oligonucleotide"
cacatcacgtcgtagtcagctgcagtcacctgtcgc

SEQ ID NO: 41 - DNA, 36 bp, Artificial Sequence
  source: /note="Description of Artificial Sequence: Synthetic oligonucleotide"
cacatcacgtcgtagtcggctgcagtcacctgtcgc

SEQ ID NO: 42 - DNA, 36 bp, Artificial Sequence
  source: /note="Description of Artificial Sequence: Synthetic oligonucleotide"
cacatcacgtcgtagtctgctgcagtcacctgtcgc

SEQ ID NO: 43 - DNA, 36 bp, Artificial Sequence
  source: /note="Description of Artificial Sequence: Synthetic oligonucleotide"
cacatcacgtcgtagtccgctgcagtcacctgtcgc

SEQ ID NO: 44 - DNA, 78 bp, Artificial Sequence
  source: /note="Description of Artificial Sequence: Synthetic oligonucleotide"
  modified_base (36)..(36): 2'-deoxyinosine
  modified_base (58)..(58): Tamra-dT
tcgactacgacgtgacttttagtcacgtcgtagtcnagctgcagtcacctgctgcttnttgcagcaggtgactgcagc

SEQ ID NO: 45 - DNA, 79 bp, Artificial Sequence
  source: /note="Description of Artificial Sequence: Synthetic oligonucleotide"
  modified_base (36)..(36): 2'-deoxyinosine
  modified_base (58)..(58): Tamra-dT
tcgactacgacgtgacttttagtcacgtcgtagtcnagctgcagtcacctgctgcttnttgcagcaggtgactgcagct

SEQ ID NO: 46 - DNA, 42 bp, Artificial Sequence
  source: /note="Description of Artificial Sequence: Synthetic oligonucleotide"
  modified_base (21)..(21): Tamra-dT phosphate
gctgcagtcacctgctgcttnttgcagcaggtgactgcagct

SEQ ID NO: 47 - DNA, 38 bp, Artificial Sequence
  source: /note="Description of Artificial Sequence: Synthetic oligonucleotide"
  modified_base (36)..(36): 2'-deoxyinosine
ccgactacgacgtgacttttagtcacgtcgtagtcnga

SEQ ID NO: 48 - DNA, 78 bp, Artificial Sequence; identical to SEQ ID NO: 44
  source: /note="Description of Artificial Sequence: Synthetic oligonucleotide"
  modified_base (36)..(36): 2'-deoxyinosine
  modified_base (58)..(58): Tamra-dT

SEQ ID NO: 49 - DNA, 38 bp, Artificial Sequence; identical to SEQ ID NO: 47
  source: /note="Description of Artificial Sequence: Synthetic oligonucleotide"
  modified_base (36)..(36): 2'-deoxyinosine

SEQ ID NO: 50 - DNA, 58 bp, Artificial Sequence
  source: /note="Description of Artificial Sequence: Synthetic oligonucleotide"
  modified_base (16)..(16): 2'-deoxyinosine
  modified_base (38)..(38): Tamra-dT
agtcacgtcgtagtcnagctgcagtcacctgctgcttnttgcagcaggtgactgcagc

SEQ ID NO: 51 - DNA, 17 bp, Artificial Sequence
  source: /note="Description of Artificial Sequence: Synthetic oligonucleotide"
tcgactacgacgtgact

SEQ ID NO: 52 - DNA, 18 bp, Artificial Sequence
  source: /note="Description of Artificial Sequence: Synthetic oligonucleotide"
  modified_base (16)..(16): 2'-deoxyinosine
agtcacgtcgtagtcnga

SEQ ID NO: 53 - DNA, 17 bp, Artificial Sequence
  source: /note="Description of Artificial Sequence: Synthetic oligonucleotide"
ccgactacgacgtgact

SEQ ID NO: 54 - DNA, 78 bp, Artificial Sequence
  source: /note="Description of Artificial Sequence: Synthetic oligonucleotide"
  modified_base (35)..(35): 2'-deoxyinosine
  modified_base (57)..(57): Tamra-dT
cgactacgacgtgacttttagtcacgtcgtagtcnagctgcagtcacctgctgcttnttgcagcaggtgactgcagct

SEQ ID NO: 55 - DNA, 37 bp, Artificial Sequence
  source: /note="Description of Artificial Sequence: Synthetic oligonucleotide"
  modified_base (35)..(35): 2'-deoxyinosine
cgactacgacgtgacttttagtcacgtcgtagtcnaa

SEQ ID NO: 56 - DNA, 78 bp, Artificial Sequence
  source: /note="Description of Artificial Sequence: Synthetic oligonucleotide"
  modified_base (35)..(35): 2'-deoxyinosine
  modified_base (52)..(52): Tamra-dT
  modified_base (57)..(57): Biotin-dT
cgactacgacgtgacttttagtcacgtcgtagtcnagctgcagtcacctgcngcttnttgcagcaggtgactgcagct

SEQ ID NO: 57 - DNA, 38 bp, Artificial Sequence; identical to SEQ ID NO: 47
  source: /note="Description of Artificial Sequence: Synthetic oligonucleotide"
  modified_base (36)..(36): 2'-deoxyinosine

SEQ ID NO: 58 - DNA, 62 bp, Artificial Sequence
  source: /note="Description of Artificial Sequence: Synthetic oligonucleotide"
  modified_base (60)..(60): 2'-deoxyinosine
acgagtgacctggttttttttttttttttttttttttttttttttttaccaggtcactcntg

SEQ ID NO: 59 - DNA, 58 bp, Artificial Sequence
  source: /note="Description of Artificial Sequence: Synthetic oligonucleotide"
  modified_base (16)..(16): 2'-deoxyinosine
  modified_base (33)..(33): Tamra-dT
  modified_base (38)..(38): Biotin-dT
agtcacgtcgtagtcnagctgcagtcacctgcngcttnttgcagcaggtgactgcagc

SEQ ID NO: 60 - DNA, 18 bp, Artificial Sequence
  source: /note="Description of Artificial Sequence: Synthetic oligonucleotide"
  modified_base (16)..(16): 2'-deoxyinosine
agtcacgtcgtagtcnaa

SEQ ID NO: 61 - DNA, 67 bp, Artificial Sequence
  source: /note="Description of Artificial Sequence: Synthetic oligonucleotide"
  modified_base (16)..(16): 2'-deoxyinosine
agtcacgtcgtagtcnagctgcagtcacctgctgcttttttttttttttgcagcaggtgactgcagc

SEQ ID NO: 62 - DNA, 67 bp, Artificial Sequence; identical to SEQ ID NO: 61
  source: /note="Description of Artificial Sequence: Synthetic oligonucleotide"
  modified_base (16)..(16): 2'-deoxyinosine

SEQ ID NO: 63 - DNA, 58 bp, Artificial Sequence
  source: /note="Description of Artificial Sequence: Synthetic oligonucleotide"
  modified_base (16)..(16): 2'-deoxyinosine
  modified_base (38)..(38): 5''-thiophosphate-Sp9-Sp9-Sp9-5-methylC
agtcacgtcgtagtcnagctgcagtcacctgctgcttcttgcagcaggtgactgcagc

SEQ ID NO: 64 - DNA, 58 bp, Artificial Sequence; identical to SEQ ID NO: 63
  source: /note="Description of Artificial Sequence: Synthetic oligonucleotide"
  modified_base (16)..(16): 2'-deoxyinosine
  modified_base (38)..(38): 5''-phosphate-Sp9-Sp9-Sp9-5-methylC

SEQ ID NO: 65 - DNA, 59 bp, Artificial Sequence
  source: /note="Description of Artificial Sequence: Synthetic oligonucleotide"
  modified_base (16)..(16): 2'-deoxyinosine
  modified_base (38)..(38): 5''-thiophosphate-Sp9-Sp9-Sp9-5-methylC
agtcacgtcgtagtcnagctgcagtcacctgctgcttcttgcagcaggtgactgcagct

SEQ ID NO: 66 - DNA, 59 bp, Artificial Sequence
  source: /note="Description of Artificial Sequence: Synthetic oligonucleotide"
  modified_base (38)..(38): 5''-thiophosphate-Sp9-Sp9-Sp9-5-methylC
agtcacgtcgtagtcgagctgcagtcacctgctgcttcttgcagcaggtgactgcagct

SEQ ID NO: 67 - DNA, 18 bp, Artificial Sequence
  source: /note="Description of Artificial Sequence: Synthetic oligonucleotide"
  modified_base (16)..(16): 2'-deoxyinosine
agtcacgtcgtagtcnaa

SEQ ID NO: 68 - DNA, 18 bp, Artificial Sequence
  primer sequence - figure 51
gcgacaggtgactgcagc

SEQ ID NO: 69 - DNA, 18 bp, Artificial Sequence
  template sequence - figure 51
gctgcagtcacctgtcgc

SEQ ID NO: 70 - DNA, 43 bp, Artificial Sequence
  source: /note="Description of Artificial Sequence: Hairpin blunt end - figure 58"
  modified_base (17)..(17): TAMRA-dT
agctgcagtcacctgcngctttttgcagcaggtgactgcagct

SEQ ID NO: 71 - DNA, 18 bp, Artificial Sequence
  source: /note="Description of Artificial Sequence: Inosine-strand - figure 58"
  modified_base (16)..(16): 2'-deoxyinosine
agtcacgtcgtagtcnca

SEQ ID NO: 72 - DNA, 18 bp, Artificial Sequence
  Helper strand - figure 58
tgcgactacgacgtgact

SEQ ID NO: 73 - DNA, 44 bp, Artificial Sequence
  source: /note="Description of Artificial Sequence: Hairpin 1 base overhang T- figure 62"
  modified_base (20)..(20): TAMRA-dT
tgctgtagtcaccatctgcntttttagcagatggtgactacagc

SEQ ID NO: 74 - DNA, 44 bp, Artificial Sequence
  source: /note="Description of Artificial Sequence: Hairpin 1 base overhang C - figure 62"
  modified_base (20)..(20): TAMRA-dT
cgctgtagtcaccatctgcntttttagcagatggtgactacagc

SEQ ID NO: 75 - DNA, 45 bp, Artificial Sequence
  source: /note="Description of Artificial Sequence: Hairpin 2 base overhang - figure 62"
  modified_base (21)..(21): TAMRA-dT
acgctgtagtcaccatctgcntttttagcagatggtgactacagc

SEQ ID NO: 76 - DNA, 46 bp, Artificial Sequence
  source: /note="Description of Artificial Sequence: Hairpin 3 base overhang - figure 62"
  modified_base (22)..(22): TAMRA-dT
cacgctgtagtcaccatctgcntttttagcagatggtgactacagc

SEQ ID NO: 77 - DNA, 47 bp, Artificial Sequence
  source: /note="Description of Artificial Sequence: Hairpin 4 base overhang - figure 62"
  modified_base (23)..(23): TAMRA-dT
tcacgctgtagtcaccatctgcntttttagcagatggtgactacagc

SEQ ID NO: 78 - DNA, 18 bp, Artificial Sequence
  source: /note="Description of Artificial Sequence: Inosine strand - figure 62"
  modified_base (16)..(16): 2'-deoxyinosine
agtcacgtcgtagtcncg

SEQ ID NO: 79 - DNA, 19 bp, Artificial Sequence
  Helper strand - overhang T - figure 62
acgcgactacgacgtgact

SEQ ID NO: 80 - DNA, 19 bp, Artificial Sequence
  Helper strand - overhang C - figure 62
gcgcgactacgacgtgact

SEQ ID NO: 81 - DNA, 20 bp, Artificial Sequence
  Helper strand - 2 base overhang - figure 62
gtcgcgactacgacgtgact

SEQ ID NO: 82 - DNA, 21 bp, Artificial Sequence
  Helper strand - 3 base overhang - figure 62
gtgcgcgactacgacgtgact

SEQ ID NO: 83 - DNA, 22 bp, Artificial Sequence
  Helper strand - 4 base overhang - figure 62
gtgacgcgactacgacgtgact